European Patent Application EP 4 450 634 A1, published October 23, 2024. Title: METHOD FOR DETECTING INTEGRATION SITE. Applicant: Nanjing GenScript Biotech Co., Ltd. The sequence listing filed with the application follows.

SEQUENCE LISTING (40 sequences)

SEQ ID NO: 1 - DNA, 30 bp, synthetic construct
  misc_feature 1..30: note = U base-modified stem-loop linker
  source 1..30: mol_type = other DNA
  modified_base 17: mod_base = OTHER; note = U
gtgcacgatgcgctagtcgcatcgtgcact

SEQ ID NO: 2 - DNA, 1279 bp, synthetic construct
  misc_feature 1..1279: note = AAVS1
  source 1..1279: mol_type = other DNA
aagcttgggagttccgcgttacataacttacggtaaatggcccgcctggctgaccgcccaacgacccccgcccattgacgtcaataatgacgtatgttcccatagtaacgccaatagggactttccattgacgtcaatgggtggagtatttacggtaaactgcccacttggcagtacatcaagtgtatcatatgccaagtacgccccctattgacgtcaatgacggtaaatggcccgcctggcattatgcccagtacatgaccttatgggactttcctacttggcagtacatctacgtattagtcatcgctattaccatggtgatgcggttttggcagtacatcaatgggcgtggatagcggtttgactcacggggatttccaagtctccaccccattgacgtcaatgggagtttgttttggcaccaaaatcaacgggactttccaaaatgtcgtaacaactccgccccattgacgcaaatgggcggtaggcgtgtacggtgggaggtctatataagcagagctcgtttagtgaaccgtcagatcgcctggccgccaccatggtgagcaagggcgaggagctgttcaccggggtggtgcccatcctggtcgagctggacggcgacgtaaacggccacaagttcagcgtgtccggcgagggcgagggcgatgccacctacggcaagctgaccctgaagttcatctgcaccaccggcaagctgcccgtgccctggcccaccctcgtgaccaccctgacctacggcgtgcagtgcttcagccgctaccccgaccacatgaagcagcacgacttcttcaagtccgccatgcccgaaggctacgtccaggagcgcaccatcttcttcaaggacgacggcaactacaagacccgcgccgaggtgaagttcgagggcgacaccctggtgaaccgcatcgagctgaagggcatcgacttcaaggaggacggcaacatcctggggcacaagctggagtacaactacaacagccacaacgtctatatcatggccgacaagcagaagaacggcatcaaggtgaacttcaagatccgccacaacatcgaggacggcagcgtgcagctcgccgaccactaccagcagaacacccccatcggcgacggccccgtgctgctgcccgacaaccactacctgagcacccagtccgccctgagcaaagaccccaacgagaagcgcgatcacatggtcctgctggagttcgtgaccgccgccgggatcactctcggcatggacgagctgtacaagtaa

SEQ ID NO: 3 - DNA, 50 bp, synthetic construct
  misc_feature 1..50: note = 3
  source 1..50: mol_type = other DNA
tcctggcagggctgtggtgaggaggggggtgtccgtgtggaaaactccct

SEQ ID NO: 4 - DNA, 50 bp, synthetic construct
  misc_feature 1..50: note = 5
  source 1..50: mol_type = other DNA
tcctccgtgcgtcagttttacctgtgagataaggccagtagccagccccg

SEQ ID NO: 5 - DNA, 17 bp, synthetic construct
  misc_feature 1..17: note = 5-RCA-AAVS1
  source 1..17: mol_type = other DNA
ggctgaccgcccaacga

SEQ ID NO: 6 - DNA, 22 bp, synthetic construct
  misc_feature 1..22: note = 5-RCA-AAVS1
  source 1..22: mol_type = other DNA
tatgtaacgcggaactcccaag

SEQ ID NO: 7 - DNA, 33 bp, synthetic construct
  misc_feature 1..33: note = Stubby Adapter-P5
  source 1..33: mol_type = other DNA
acactctttccctacacgacgctcttccgatct

SEQ ID NO: 8 - DNA, 33 bp, synthetic construct
  misc_feature 1..33: note = Stubby Adapter-P7
  source 1..33: mol_type = other DNA
gatcggaagagcacacgtctgaactccagtcac

SEQ ID NO: 9 - DNA, 19 bp, synthetic construct
  misc_feature 1..19: note = Universal-F
  source 1..19: mol_type = other DNA
tacacgacgctcttccgat

SEQ ID NO: 10 - DNA, 40 bp, synthetic construct
  misc_feature 1..40: note = AAVS1
  source 1..40: mol_type = other DNA
acgtgtgctcttccgatctgggccatttaccgtaagttat

SEQ ID NO: 11 - DNA, 62 bp, synthetic construct
  misc_feature 1..62: note = P5
  source 1..62: mol_type = other DNA
aatgatacggcgaccaccgagatctacacacactctttccctacacgacgctcttccgatct

SEQ ID NO: 12 - DNA, 57 bp, synthetic construct
  misc_feature 1..57: note = P7
  source 1..57: mol_type = other DNA
caagcagaagacggcatacgagatgtgactggagttcagacgtgtgctcttccgatc

SEQ ID NO: 13 - DNA, 131 bp, synthetic construct
  misc_feature 1..131: note = Chr19
  source 1..131: mol_type = other DNA
ctttggctcttcacctttctagtccccaatttatattgttcctccgtgcgtcagttttacctgtgagataaggccagtagccagccccgaagcttgggagttccgcgttacataacttacggtaaatggcc

SEQ ID NO: 14 - DNA, 137 bp, synthetic construct
  misc_feature 1..137: note = Chr4
  source 1..137: mol_type = other DNA
aactttatgagctgtaacactcaccatgaaggtctgcagcttcactcctccgtgcgtcagttttacctgtgagataaggccagtagccagccccgaagcttgggagttccgcgttacataacttacggtaaatggcc

SEQ ID NO: 15 - DNA, 165 bp, synthetic construct
  misc_feature 1..165: note = Chr1
  source 1..165: mol_type = other DNA
aaagaactatttatgatattcgtggatctgtagatcagaaattggggtggggcacagtgaggagggtgtccgttcctccgtgcgtcagttttacctgtgagataaggccagtagccagccccgaagcttgggagttccgcgttacataacttacggtaaatggcc

SEQ ID NO: 16 - DNA, 157 bp, synthetic construct
  misc_feature 1..157: note = Chr3
  source 1..157: mol_type = other DNA
ggtttctctctctctctccattagcttttgctgttcacccaaatagactctccagtttatattgttcctccgtgcgtcagttttacctgtgagataaggccagtagccagccccgaagcttgggagttccgcgttacataacttacggtaaatggcc

SEQ ID NO: 17 - DNA, 150 bp, synthetic construct
  misc_feature 1..150: note = Chr6
  source 1..150: mol_type = other DNA
gtgttctaaagtgtaaacgatgaatatggatactttggctgtttacacagcctgaatatcctccgtgcgtcagttttacctgtgagataaggccagtagccagccccgaagcttgggagttccgcgttacataacttacggtaaatggcc

SEQ ID NO: 18 - DNA, 137 bp, synthetic construct; identical to SEQ ID NO: 14
  misc_feature 1..137: note = Chr2
  source 1..137: mol_type = other DNA

SEQ ID NO: 19 - DNA, 150 bp, synthetic construct
  misc_feature 1..150: note = Chr7
  source 1..150: mol_type = other DNA
ccccgagtccctcctcctgtgctctgagtccctatttctgtgccccaatttatattgttcctccgtgcgtcagttttacctgtgagataaggccagtagccagccccgaagcttgggagttccgcgttacataacttacggtaaatggcc

SEQ ID NO: 20 - DNA, 150 bp, synthetic construct
  misc_feature 1..150: note = Chr20
  source 1..150: mol_type = other DNA
cagtggtggcagttgcccatgcagggcagcgcatggagactccagtcagccagccccgtcctccgtgcgtcagttttacctgtgagataaggccagtagccagccccgaagcttgggagttccgcgttacataacttacggtaaatggcc

SEQ ID NO: 21 - DNA, 20 bp, synthetic construct
  misc_feature 1..20: note = Chr19
  source 1..20: mol_type = other DNA
cgatggagccagagaggatc

SEQ ID NO: 22 - DNA, 20 bp, synthetic construct
  misc_feature 1..20: note = Chr19
  source 1..20: mol_type = other DNA
gtcccgttgattttggtgcc

SEQ ID NO: 23 - DNA, 771 bp, synthetic construct
  misc_feature 1..771: note = Chr19:55115264
  source 1..771: mol_type = other DNA
cgatggagccagagaggatcctgggagggagagcttggcagggggtgggagggaagggggggatgcgtgacctgcccggttctcagtggccaccctgcgctaccctctcccagaacctgagctgctctgacgcggctgtctggtgcgtttcactgatcctggtgctgcagcttccttacacttcccaagaggagaagcagtttggaaaaacaaaatcagaataagttggtcctgagttctaactttggctcttcacctttctagtccccaatttatattgttcctccgtgcgtcagttttacctgtgagataaggccagtagccagccccgaagcttgggagttccgcgttacataacttacggtaaatggcccgcctggctgaccgcccaacgacccccgcccattgacgtcaataatgacgtatgttcccatagtaacgccaatagggactttccattgacgtcaatgggtggagtatttacggtaaactgcccacttggcagtacatcaagtgtatcatatgccaagtacgccccctattgacgtcaatgacggtaaatggcccgcctggcattatgcccagtacatgaccttatgggactttcctacttggcagtacatctacgtattagtcatcgctattaccatggtgatgcggttttggcagtacatcaatgggcgtggatagcggtttgactcacggggatttccaagtctccaccccattgacgtcaatgggagtttgttttggcaccaaaatcaacgggac

SEQ ID NO: 24 - DNA, 635 bp, synthetic construct
  misc_feature 1..635: note = LTRs
  source 1..635: mol_type = other DNA
tggaagggctaattcactcccaaagaagacaagatatccttgatctgtggatctaccacacacaaggctacttccctgattagcagaactacacaccagggccaggggtcagatatccactgacctttggatggtgctacaagctagtaccagttgagccagataaggtagaagaggccaataaaggagagaacaccagcttgttacaccctgtgagcctgcatgggatggatgacccggagagagaagtgttagagtggaggtttgacagccgcctagcatttcatcacgtggcccgagagctgcatccggagtacttcaagaactgctgatatcgagcttgctacaagggactttccgctggggactttccagggaggcgtggcctgggcgggactggggagtggcgagccctcagatcctgcatataagcagctgctttttgcctgtactgggtctctctggttagaccagatctgagcctgggagctctctggctaactagggaacccactgcttaagcctcaataaagcttgccttgagtgcttcaagtagtgtgtgcccgtctgttgtgtgactctggtaactagagatccctcagacccttttagtcagtgtggaaaatctctagcag

SEQ ID NO: 25 - DNA, 22 bp, synthetic construct
  misc_feature 1..22: note = 5-RCA-LTRs
  source 1..22: mol_type = other DNA
cacaaggctacttccctgatta

SEQ ID NO: 26 - DNA, 23 bp, synthetic construct
  misc_feature 1..23: note = 5-RCA-LTRs
  source 1..23: mol_type = other DNA
tatcttgtcttctttgggagtga

SEQ ID NO: 27 - DNA, 17 bp, synthetic construct
  misc_feature 1..17: note = Universal-F
  source 1..17: mol_type = other DNA
cacgacgctcttccgat

SEQ ID NO: 28 - DNA, 39 bp, synthetic construct
  misc_feature 1..39: note = LTRs
  source 1..39: mol_type = other DNA
acgtgtgctcttccgatctcttgtcttctttgggagtga

SEQ ID NO: 29 - DNA, 56 bp, synthetic construct
  misc_feature 1..56: note = NW_003613601.1
  source 1..56: mol_type = other DNA
acttttctctggaaatggctttgtggaagggctaattcactcccaaagaagacaag

SEQ ID NO: 30 - DNA, 178 bp, synthetic construct
  misc_feature 1..178: note = NW_003614821.1
  source 1..178: mol_type = other DNA
aatgatacccaaatctcgggctaagttctcccgaccttcaagaccttgaagctagaaaaaaagatttaggtgtggaaaatatagcagaagcagtcaggtgagaaagaattttagggacttaaagacatctctaaagtcaaagaggtggaagggctaattcactcccaaagaagacaag

SEQ ID NO: 31 - DNA, 150 bp, synthetic construct
  misc_feature 1..150: note = NW_003614611.1
  source 1..150: mol_type = other DNA
atgtatacacttaatattctccaagattgaagagtggagatctattacttactaggtttcttatttgtcagcttcatgatttcttcagagtgttttttttaaaactttgttcgtaattggaagggctaattcactcccaaagaagacaag

SEQ ID NO: 32 - DNA, 175 bp, synthetic construct
  misc_feature 1..175: note = NW_003613734.1
  source 1..175: mol_type = other DNA
taccctgtgccattctgaaggaaattcaggtttggagaagttaggtaatttgtttcacaagaccacacagctaaatgagaagcactgagattcaagcccaggactatctgtgaccagtgttctccccagcccttgccatgtctggaagggctaattcactcccaaagaagacaag

SEQ ID NO: 33 - DNA, 151 bp, synthetic construct
  misc_feature 1..151: note = NW_003614154.1
  source 1..151: mol_type = other DNA
ctcatcttatttgttaattcaattttgaaattgtttaaactcatacaccaaacatacacatattgtttgtaattcttaccattcttagacttgtcagcaaatcactgttctgtgatactggaagggctaattcactcccaaagaagacaag

SEQ ID NO: 34 - DNA, 158 bp, synthetic construct
  misc_feature 1..158: note = NW_003613767.1
  source 1..158: mol_type = other DNA
tatttgtatagtatatacgaagagtagaagactatggtgttattttgccccttatctctaaaggcttattcttgagatatcaacacgtgggtctatgtatattgatacagatattatggaatgtttggaagggctaattcactcccaaagaagacaag

SEQ ID NO: 35 - DNA, 179 bp, synthetic construct
  misc_feature 1..179: note = NW_003613592.1
  source 1..179: mol_type = other DNA
atttctattaccaattaattccttattaatgattcttggagtttcaatctgctctttaactattcactatcgtagctccaggtagtaaaactaaaaacatttcttgctaattccaatgaacgtgtctttctctggaaatggctttgtggaagggctaattcactcccaaagaagacaag

SEQ ID NO: 36 - DNA, 160 bp, synthetic construct
  misc_feature 1..160: note = NW_003615763.1
  source 1..160: mol_type = other DNA
gtgtgtgtgtgtgtgtgtgtgtgtgtgtggacatgtggatgcaggtacatgtgtgtgtatatggagagggcagatgtcaatctctggtttcttccacaggcaccatctactctatcttttgagatagtggaagggctaattcactcccaaagaagacaag

SEQ ID NO: 37 - DNA, 164 bp, synthetic construct
  misc_feature 1..164: note = NW_003613979.1
  source 1..164: mol_type = other DNA
gagatataacagcagatgtgacagtcataataagaaagtgtacaggctacttctttaaattacaagaaatgagaagcaagaacagttaacatttccaaaatgggactttttatagctgtggtgtcctttagtggaagggctaattcactcccaaagaagacaag

SEQ ID NO: 38 - DNA, 992 bp, synthetic construct
  misc_feature 1..992: note = NW_003614611.1
  source 1..992: mol_type = other DNA
agtatgatagtgtgtgtgtgtgtgtgtgtgtgtgtgtgtgtgtgtgtgtgcatgtgtgtgtttgtcctcaatctatgtacatgcttatgtgtgctagtgtttatgtatgataatttcaatttcctacagtttcttgaatgtcaggcaacagccatggatcttggttttcctattctgccttgacagaggcagtgtcccttactgtttattgcttacacagtaaaatcctgtgccctgtgaaccctgttttcagccaccttatatcattcttaaatgcttcattatctgaattttttatttctcaaagtatcaacatgattgaacttctcaactagggcattaacatgcaagaaaagacaaaatacctgtggcttgcagaggttcatctttccaatgtaattgatatccatataacatctcatttataaatcaaccatgctcactaggaaataataatcttaattttaattaatttatttttatttaaattagattattctctcaaacaatagaaaaagattttttaaatgcttcaggtttgtgtttgtttaattactctttagaataaatttttctacagaaagtactcaattttttattttgagctaaaaactttcagataagtcaaggtcttgagttttctctattagtacaaaacagggggattagagtttaatgtatacacttaatattctccaagattgaagagtggagatctattacttactaggtttcttatttgtcagcttcatgatttcttcagagtgttttttttaaaactttgttcgtaattggaagggctaattcactcccaaagaagacaagatatccttgatctgtggatctaccacacacaaggctacttccctgattagcagaactacacaccagggccaggggtcagatatccactgacctttggatggtgctacaagctagtaccagttgagccagataaggtagaagaggccaataaaggagagaacaccagc

SEQ ID NO: 39 - DNA, 20 bp, synthetic construct
  misc_feature 1..20: note = NW_003614611.1
  source 1..20: mol_type = other DNA
tcccttactgtttattgctt

SEQ ID NO: 40 - DNA, 19 bp, synthetic construct
  misc_feature 1..19: note = NW_003614611.1
  source 1..19: mol_type = other DNA
gctggtgttctctccttta